European Patent Application EP 4 806 990 A1, published September 16, 2026. Title: 一种细胞株及其制备方法与应用. Applicant: 深圳太力生物技术有限责任公司. The sequence listing filed with the application follows.

SEQUENCE LISTING (9 sequences)

SEQ ID NO: 1 - DNA, 444 bp, synthetic construct
  source 1..444: mol_type = other DNA
taattctggcaactatcaaaggttcaccaaggaaggaattctttatttggtatctgcaagcgcctgggtgttccaatttctatctgcaaatgtttgttcctgcagacatgtctaactatggtggaaacagagaccagcctcagatgtcacactgtgacctgacctataaaagctgaactttacaaagcataagcttgggttcatgcctgagtgaaaccagactgagtttctcttgtctctccgactgcttgcttggtcctgtgctggctaaaatttccatgacagtaggggtgtaaattattcagttttagtttcccagaaaactaaaagtaagactgtcatatgacctaatgatttgacttctggggtcctttcaattagctgttgaaaggacaatagattactcatggccatttaaacaattcacagtagcaaaaaggtgag

SEQ ID NO: 2 - DNA, 642 bp, synthetic construct
  source 1..642: mol_type = other DNA
caaccaggtctaactcaaccaccaagtgtgtctgtcgccccaggacaaaccgccagaatcacctgtggcggcaacaacatcggctctaagtccgtccattggtatcagcagaagcctggtcaggcccccgtgctcgtggtgtacgacgactccgaccggcctagcggcatccccgagcggttctccggctccaactccggcaataccgctaccctgaccatctccagagtggaagctggcgatgaggccgattactactgccaggtgtgggactctagctctgatcactacgtgttcggcaccggcaccaaagtgaccgtgctgtcctccgcctctacaaagggcccatctgtttttcctctggctccttcctccaagtctacctctggcggaacagctgctctgggctgcctggtgaaggactacttccctgagcctgtgactgtgtcctggaacagcggagccctgacctccggcgtgcacaccttccctgccgtgctgcagtcctctggcctgtactccctgtcttccgtggtcaccgtgccttcttctagcctgggcacccagacctacatctgcaacgtgaaccacaagcccagcaacacaaaagtggacaagaaggtggaacctaagtcctgctaa

SEQ ID NO: 3 - DNA, 1392 bp, synthetic construct
  source 1..1392: mol_type = other DNA
caagtgcaactagtgcaaagtggtgcagaagtgaagaagcctggcgcttctgtcaaggtttcttgcaaggccagcggctacaccttcaccggctattacatgcactgggtcagacaggcccccgggcagggcctggaatggatgggctggatcaaccctaactccggaggcacaaattacgctcagaagtttcagggcagagtgaccatgacccgggatacctccatctccacagcttacatggaactgagcaggctgagatccgacgacaccgctgtgtactactgcgccagatcccccaatccttactactacgactcctccggctactactacccaggcgccttcgacatctggggacaaggcaccatggtcaccgtgagctctgcctccgtggccgctccgtccgtgttcatcttccccccctctgacgagcaactgaagtccggcaccgcttccgtcgtctgtctgctgaacaacttctatcctcgggaggccaaagtgcagtggaaggtggacaacgctctgcagtctggcaattctcaagagtctgtgaccgagcaggatagcaaggactccacctactccctctctagcaccctgaccctgtccaaagccgactacgagaagcacaaggtgtacgcctgcgaggtgacccaccagggactgtcctctcctgtgacaaaatcttttaaccggggagagtgcgacaagacccacacctgccctccttgtcctgctcccgagttgctgggcggccctagtgtgtttctgttccctcctaagcccaaggatacactgatgatctctcggaccccagaagtgacctgtgtggtggtggacgtgtcccacgaggaccctgaggtgaagttcaactggtacgtggatggcgtggaagtgcacaacgccaaaaccaagcctcgggaagagcagtataacagcacatacagagtggtgtccgtgctgaccgtgctgcatcaggactggctgaacggcaaagagtacaagtgcaaggtgagcaacaaggccctgcccgcccctatcgagaagaccatctccaaggctaagggccagcctcgcgaacctcaggtgtgcacactgcctccttcaagagacgagctgaccaagaaccaggtgtctctgtcttgtgccgtgaaaggcttctacccttccgatatcgccgttgagtgggagtccaacggacagcctgaaaacaactacaagaccacccctccagtgctggactccgacggctctttcttcctcgtgtctaagctgaccgtggataagtccagatggcagcagggcaacgtgttctcttgctccgtgatgcatgaagctctgcacaaccactacacacagaaatctctgtccctgtctccaggcaagtaa

SEQ ID NO: 4 - DNA, 645 bp, synthetic construct
  source 1..645: mol_type = other DNA
gatatccaaatgactcaaagtccaagtagtctctccgccagcgtcggcgacagagtgacaatcacctgttctgcttctcaggacatctccaactacctgaattggtatcagcagaagcctggcaaggcccctaaggtgctgatctacttcacctcctctctgcactctggcgtgccctcccggttctccggctctggatctggcaccgattttaccctgaccatcagcagcctgcagcctgaagattttgctacctactactgccagcagtactctaccgtgccttggaccttcggccagggaacaaaagtcgagatcaagcggactgtggccgctccttctgtgttcatcttccctccatccgacgagcagctgaagtctggcaccgccagcgtggtgtgcctgctgaacaacttctaccccagagaggccaaggtgcagtggaaggtggacaacgccctgcagtccggcaactcccaagagtccgttaccgaacaggattccaaggactccacctattccctgtcttccaccctgacactgtccaaagctgactacgagaagcacaaggtgtacgcctgcgaagtgacccatcaaggcctgtctagccctgtgaccaagtccttcaacagaggcgagtgctaa

SEQ ID NO: 5 - DNA, 1362 bp, synthetic construct
  source 1..1362: mol_type = other DNA
gaagtgcaactagtggaaagtggtggtggtctcgtgcagcctggcggcagcctgagactgtcttgtgccgcttctggctacaccttcaccaactacggcatgaactgggtgcggcaggctcccggcaagggactggaatgggtcggctggatcaacacctataccggcgagcccacctacgccgccgacttcaagcggcggttcacattcagcctggatacctccaagtctacagcctacctgcagatgaatagcctgagagccgaggacaccgctgtgtactactgcgctaagtaccctcactactacggcagctcccactggtatttcgacgtgtggggccagggcaccctggtcacagtctcttctgcctccaccaaaggcccttccgtgttccctctggccccatcatctaaatctacctccggcggcaccgctgccctgggctgtctggtgaaggactacttcccagaacctgtgaccgtgtcctggaactccggcgctctgacttctggcgtgcacacctttcctgccgtgctgcagtcctctggtctatactctctgtcctccgtggtgacagtgccttccagctctctgggaacacagacctacatctgtaacgtgaaccacaagccctccaacacaaaggtggataagaaggtcgaacccaagtcctgtgacaagacccacacctgccctccttgccctgctcctgaactgctgggaggcccttccgtgtttctgtttcctcctaagcccaaagatacactgatgatcagccgcaccccagaagtgacctgcgtggtcgtggacgtgtctcacgaggaccctgaggtgaagttcaactggtacgtggatggcgtggaagtgcacaacgccaagaccaagcctagagaggaacagtacaactccacctacagagtggtgtccgtgctgaccgtgctgcatcaggactggctgaacggcaaagagtacaagtgcaaggtgtctaacaaggccctgcccgctcctatcgagaagaccatctctaaagctaagggacaacctcgggagcctcaagtgtataccctgcctccctgcagagacgagctgaccaagaaccaggtgtccctgtggtgcctggtgaagggcttctaccccagcgacatcgccgtcgagtgggagtccaatggccagcctgagaacaactacaaaaccacccctccagtcctggactctgacggctctttcttcctgtactccaagctgaccgtggacaagtccagatggcagcagggcaacgttttctcctgctctgtgatgcacgaggccctgcacaatcattacacccagaagtccctgtccctctctcctggcaagtaa

SEQ ID NO: 6 - protein, 22 aa, synthetic construct
MDMRVPAQLLGLLLLWLRGARC

SEQ ID NO: 7 - protein, 19 aa, synthetic construct
MGWSCIILFLVATATGVHS

SEQ ID NO: 8 - DNA, 303 bp, synthetic construct
  source 1..303: mol_type = other DNA
acaaagggcccatctgtttttcctctggctccttcctccaagtctacctctggcggaacagctgctctgggctgcctggtgaaggactacttccctgagcctgtgactgtgtcctggaacagcggagccctgacctccggcgtgcacaccttccctgccgtgctgcagtcctctggcctgtactccctgtcttccgtggtcaccgtgccttcttctagcctgggcacccagacctacatctgcaacgtgaaccacaagcccagcaacacaaaagtggacaagaaggtggaacctaagtcctgc

SEQ ID NO: 9 - DNA, 315 bp, synthetic construct
  source 1..315: mol_type = other DNA
gtggccgctccgtccgtgttcatcttccccccctctgacgagcaactgaagtccggcaccgcttccgtcgtctgtctgctgaacaacttctatcctcgggaggccaaagtgcagtggaaggtggacaacgctctgcagtctggcaattctcaagagtctgtgaccgagcaggatagcaaggactccacctactccctctctagcaccctgaccctgtccaaagccgactacgagaagcacaaggtgtacgcctgcgaggtgacccaccagggactgtcctctcctgtgacaaaatcttttaaccggggagagtgc